European Patent Specification EP 3 317 402 B1, published February 14, 2024. Title: A VIABLE CELL POPULATION, METHOD FOR PRODUCTION AND USES THEREOF. Applicant: Stemlab, S.A. The sequence listing filed with the application follows.

SEQUENCE LISTING (2 sequences)

SEQ ID NO: 1 - protein, 25 aa, Homo sapiens
  gp100 long peptide
YLEPGPVTANRQLYPEWTEAQRLDC

SEQ ID NO: 2 - protein, 9 aa, Homo sapiens
  gp100 short peptide
YLEPGPVTA